European Patent Application EP 4 538 367 A2, published April 16, 2025. Title: Polypeptides for Use in the Synthesis of Kratom Alkaloids. Applicant: Mitradyne Corporation. Application US. The sequence listing filed with the application follows.

SEQUENCE LISTING (65 sequences)

SEQ ID NO: 1 - protein, 509 aa, Mitragyna speciosa
MSTPPTKFSGTLSRSDFPEGFLFGSASSAFQYEGAHNVDGRLPSIWDTFLKETHPDIVAANGLDAVEFYYRYREDIKAMKDIGLDTFRFSLSWPRILPNGRRTKGPNNEEQGVNRLAIDFYNTVINLLLENGIEPSVTLFHWDLPQALETEYLGFLSQKSVEDFVDYADLCFREFGDRVKYWMTFNETWSYSLFGYLLGTFAPGRGSTDEGQRRAMAEVLPSSLGRSKQAFAHSRTPRAGDPTTEPYIVTHNQLLAHAAATKLYRREYQNVQKGKMGIGLVTIWTEPHTDTQEDRDAAQRVLDFMLGWLFDPVVFGKYPESMRRLVGNRLPEFTPEQSRDLIGSFDFIGMNYYTANSVANRPYSRSIIYNPDSQAICFSLGEEAGSSWVYIYPQGLLKLLLYVKEKYNNPVIYITENGIDEVNDENLTMWEALYDTQRISYHKQHIEATKQAISQGADVRGYYAWSFTDNLEWASGFDSRFGLNYVHFGRELERYPKLSAGWFKFFLDK

SEQ ID NO: 2 - protein, 544 aa, Mitragyna speciosa
MAASNVLSPISRADFGEEFIFGSASSAYQMEGAAAEGGRGPSIWDTFTEQTPDKVMDGSNGNVAINQYYLYKEDVKLMKKIGLDAYRFSISWPRVLPGGRLSAGVNKAGIDYYNNLINELLANDIKPFVTLFHWDVPQALEDEYGGFLNRKIVNDFREFAELCFWEFGDRVKNWITLNEPWSFAFGGYTTGAYAPGRGAATPEHMKDAIPKHRCHCLHQVGDCQAGDPGTEPYLVAHHLLLAHAEAVKLYREYFQAQGGKIGITLVSQWWEPLNDTPEDKEALERAADFMFGWFMSPVTFGDYPKRMRDIVKSRLPKFSEEESESLRKSYDFLGLNYYTSQYVTDASGTKSDLVSYVTDQQVKTQVVGPDGKTEIGPQAGSSWLYIYPIGIYKVLKYIKSHYDDPIIYITENGVDELNDLKVTVSKGRADKIRIKYHHDHLEYVKQAMDVDKVKVKGYFIWSLLDNFEWAEGFAVRFGIIHVNYKDGYARYPKESAIWFMKFLNKSIGNEPSQPTKPTKRALSNGDLEANSNVEEIPKKKVLKF

SEQ ID NO: 3 - protein, 546 aa, Mitragyna speciosa
MEIRRSDFGQNFLFGSATAAYQIEGATEEGGRRPSIWDTMIRRHPDRISNYDDAKVAIDSYHLYKDDVKFMKQIGLDAYRFSISWTRVLPGGRLNAGVNKEGIKYYNNLINELLAHGIQPFVTLFHFEVPQALEDEYGGFLSDKIVKDFSEFAGLCFWEFGDRVKHWTTLNEPWTFANYGYAVGSFPPNRGSSSADHASVPIVQHRSDRTSAQICENGDPGREPYIVAHNLLLAHAEAVRIYREKFKETQCGKIGITLVTHWFEPLNDTEDDKEAAKRAFDFKFGWFMEPVTYGRYPKRMTDNVPSDRLKPLTAEESAKLKGSYDFLGLNYYTATYATNDPSVKGPPSYLTDWHVKTQTTATDGKTLIGQSTSSGWIYVYPTGIYKLLSKIKAYYNDPPIFITENGVTDAGDPEGKIANGRVDEIRINYHREHLKEVKHAINENGVDVKGYFLWSLVDNFEWTAGYKDRFGIVYIDYNDPGRTRYPKESAIWFMNFLKKKKDLSTDNEETNGVAAHNTQELSQSKLQASAKDLPNNEAPAKRARKR

SEQ ID NO: 4 - protein, 502 aa, Mitragyna speciosa
MAMQVTFLLGILLLSVHLSNASSDKAAFNRKSFPDGFVFGASSAAYQYEGAAFEGGKGPSIWDTFTHEFPGKILNGSNGDVADNFYHLYKDDVKLMKFIGMDAFRFSISWPRVLPRGKLSGGVNKEGVAFYNNLINELISNGIKPFVTIYHWDTPQTLEDEYRSFLSPLIIDDYLDFVELCFKEFGDRVKHWITMNEPYIFINGGYDGGTQAPGRCSAWLANDCPAGNSATEPYIVGHHMLLCHAAAVNLYKQKYQKTQKGEIGITLVSHWVVPYTSSKLDVMATQRALDFMYGWFIHPLIYGDYPRSMRAIVKKRLPTFTTEQVKMVKGSFDFIGLNYYTAKYAANVATSNSINVSSSTDTLANLTSERNGKPIGDPTGVSIFFVYPKGLRDLLAYTKKNYNNPPIYITENGIGDANNSTLIKGIKDAQRVDFYHRHLLAVQEAIKLGVNVKGFFAWSFLDTFEWASGYTLRFGLCYVDYKDGLKRYPKSSALWFKKFLRR

SEQ ID NO: 5 - protein, 530 aa, Mitragyna speciosa
MATPESHVFPSDSPLKRQDFPEGFIFGASASAFQYEGAVDQDGRGPSIWDTFLEEKYPDIVKDGGLEAIQHYYQYKDDVQVIKETGLDIYRFSISWPRILPMGRRIVPEVGERMIEDGINEAGIEFYNGLINKLLANGIEPMVTLYHWDVPQALEDEYLGFLDKRIVCDFADYADLCFSRFGDRVKYWITFNEPWSFSVGGYSMGTFAPGRGASSNERAQMIFDFPTSRATSKQASMATGAPKEGNPGTEPYIVSHHQLLAHAAAVKLYREKYQREQGGKIGITLVSNWTVPYHDTKEDKDAAQRALDFMFGWFMDPITYGDYPSTMRSLVGNRLPLFTPIESELLVGSFDFLGFNYYTANYVKNAPNYESDAHYKLDSQAECTPVRDNVPIGEQAASDWLYVYPKGILEHVDYIREKYNNPIIYITENGRDELNQPELSYWVSLFDHKRISYHYRHLQFLKKAIANGANVEGYFVWSLMDNLEWSSGFKTRFGMNFIDFKNGLKRYPKLSSGWFKFFLHEDVQPKAEEL

SEQ ID NO: 6 - protein, 533 aa, Mitragyna speciosa
DDGSDDDDGSSGGQGGSYIIRHFNRSSFPTDFIFGAATSAFQIEGGSDRRGTNIWDVFIENNPELIANKSDAKVAADSYHRFKEDVSLLSGLGFDAYRFSISWTRLLPTGRISGGINGDGVRYYHALIDEIISKGMIPFATIFHWDLPQALEDEYKGFLSEKIVEDFARYSELCFFLFGKKVKHWITLNEPWSYTTLGYAYGAFPPNRCSKSDTLKGSGNSGFSVGRFASYNSQDGCKYGNSGTEPYIVTHHMLLAHATAVKIYRENYQKDQGGQIGITLVTQWFEPYNPKMKTDVDAAARSLAFMFGWYMDPLFTGAYPTEMVTYVDGDRLPSFKDHEAKIVKGSYDFIGLNYYTAEYSQDIPCDKSQQNYLTDPCVNPNKTRNGKPIGGKTGADWLYVYPKGFHELLVYIKDKYNNPPIYVTENGVCRDNRGPRPHDMLRVNYHRGHLMKLRFCLNRKDVNVKGYFVWSLMDNFEWLDGYFVNFGLVRIDYDNKSLNRSCKDSASWFNVFLNKDGGSNEAQICKLFPSSEN

SEQ ID NO: 7 - protein, 541 aa, Mitragyna speciosa
MAIKFFVIVSLLAFAHCAFANTSNCTCDCTGKKITRGSFPPDFVFGAASSAYQTEGAWNVSGKGPSIWDTFTHLYPEKIAFNGTYSSNGDVAIDGYDRYESDTDIIRDLGLDVYRISISWSRILPKGQISGGVNPDGIRYYNDVLNALVDKGVEPCVTVFHWDVPQALEDLYGGFLSPRIVEDFRNYADVLFKNFGDRVRTWITLNEPWSFSRYAYDLGMLAPGRCTYWDNPDCTGGDSATEPYLVTHHQLLAHAATVDLYRKNYQAKYNGLIGITIVSQWYLPYRAGNPYDELAAQIALDFMYGWFMDPITFGRYPLSMQEKVGSRLPQFTEEESRKLIHSYDFVGVNYYTATFAHFYDEGYKPPYVSYGTDSRVNLTDVDSEGKPCGKGPAGASWLQVYPLGLREILNYTKTVYDNPSIFITENGLCTNTSISKNESIHDDIRTSYLEDHLCCLLEAIDKYKVNVSGYIVWSLFDNFEWASSYEDRFGIYFVDYEDNLTRIEKDSAAWYKGVVAKSPPPPSPILIREIPSISNRKMLPA

SEQ ID NO: 8 - protein, 503 aa, Mitragyna speciosa
MVVLRRGIVLVVLVAVLGLQTCLGQINRRSFPKGFVFGTASSAYQYEGAVKVDGRGPTIWDKFAHSFGKVLDFSNADVAVDQYHLYSEDVQLMKDMGMDAYRFSIAWTRLFPNGTGELNQAGVDHYNNIINTLIASGIEPYVTIYHWDLPQALDDKYSGWLSPQIVNDFAVYAETCFQKFGDRVKHWITVNEPHTFAVQGYDVGLQAPGRCSILLRAFCRAGNSATEPYIVGHNVLLAHSTVVDIYKKKYKPMQKGSIGITLDTFWYEPASNSTEDIQATQRAIDFNLGWFLEPLIVGDYPSSMRTRVGNRLPKFSQAQSLALKGAFDFVGINHYTTWYAKNKSTSIIGVLLNDSLSDSGAITLPFKGLTPIGDRANSIWLYIVPHGIRSLMNYIKQTYGNPLVIITENGMDDGNSPFNSIQDALKDEKRIKYHNDYLTNLLAAIREDRCNVQGYFVWSLLDNWEWGAGFSSRFGLYYVDFNDKLKRYAKDSVKWFKNFLSAA

SEQ ID NO: 9 - protein, 397 aa, Mitragyna speciosa
PQALEDKYGGFLSSQIVDDFREYVELCFWEFGDRVKHWITLNEPWSFSVGGYVNGTFAPGRGASSSEQENDHPAPALLSRCSPWQSQSISSNGNPGTEPYVVTHNQLLAHAAAVELYKSNFQKSQNGKIGITLVSQWMEPLDENSKADVEAAKRALDFMLGWFMEPLTTGDYPKTMRKLVGSRLPKFSAEQSKQLKGSYDFLGLNYYTADYVTSASSSTTGGNLSYTTDSQVTHTTDRNGVPIGPQGGSEWLHIYPEGIRKLLVYVKKTYNVPLIYITENGVDEVNDTSLTLSEARVDNTRIKYIQDHLLNIRLAIGDGVNVKGYFVWSLLDNFEWSEGYTVRFGFIHIDYTNNFARYPKDSAIWFMNSFHKEYPKQFLKRTLEDHEDFVSKKRLRQ

SEQ ID NO: 10 - protein, 542 aa, Mitragyna speciosa
MALVNCILPMTNASLKPPSLHLSSLGREHQIFKANVELSSRATPRTKSNSLRINCLKGVAFPEAETISKLINGVLTSSTASTTDTQVISRKDFPTDFKFGCSTSALQTEGSGTEGGRGPSTWDDFIGTGKKAVDSYNRYKEDVKLLKDMGADCYRFSISWSRLLPDGTISGGINQEGIKFYNNFIDELISNGITPFVTLFHFDLPSALQKKYNGFLDSKIVDDFKAYADLCFKTFGDRVKYWITINEPQVFGQYGYKMQLSIPDVVTYPYTAIHNIILSHATAAKHYQQNYQPTQKGEIGISLVTEWFEAGSDTKPDKDASERAFDFLTGWMLEPLVFGDYPFIMKALVRNDLPKFTDEQKTLIKGSYDFIGVNYYTSRYATAVSLTLDEKYTSLDQYQHVTLSVYKDGKLIGEKAPGSSEIYVYPPGLGKALAYISKFYNNPKIYITENGYPEKRDDSIPQATAIKDDARIQHITAHLQSVKEAMKLGANVKGYCMWSLMDCLEMGSAYNVRYGLCYTDYSTLNRYPKKSSEWLKTFVSSK

SEQ ID NO: 11 - protein, 521 aa, Mitragyna speciosa
MKMVSKTSSSRMLLLLLITAFAALSQCAANAEELEFLNEEKLHFNTPKGLLRKSFPKGFVFGTATSAYQVEGMADKDGRGPSIWDIFIKAPGREPNNATGEVAVDQYHLYKKDVDLMKRLNFDAYRFSISWPRIFPNGSGKVNWKGVAYYNRLINYMLKQGITPYANLNHYDLPQALQDRYNGWLGREVVKDFADYADFCFKTFGDRVKNWFTFNEPRVVAALGYDNGFFAPGRCSKAFGNCTAGNSATEPYIVAHNLILCHASAVQRYREKYQEKQKGKIGILLDFVWYEPHTDTEDDKAAAQRARDFHIGWFMHPLVYGEYPKNLQNIVADRLPKFTKEEVKIVKGSFDYVGVNQYTAYYMYDPHQGKPKDIGYQQDWNCGFTYDRKGVPIGPRAYSYWLYNVPWGLYKAVMYVKENYQNPTIILAENGMDDPGNLTLPAGLKDTTRINYYKAYLAELRKTIDDGANVIGYFAWSLLDNFEWRLGYTSRFGIVYVDFKTLKRYPKMSALWFQKLLYRQP

SEQ ID NO: 12 - protein, 516 aa, Mitragyna speciosa
MSSFNLLLVFPVPFFAITSILSTQYWWVPAWGADDYVRADFPADFVFGCGTSAYQVEGAAFEDGRTPSIWDTFVHSGLVDEGNGDIACDEYHKYKEDVELMAEMGLEGYRFSISWSRLIPNGRGPVNPKGLQYYNNLINGLISRGIQPYVTLYHVDTPQALEDEYGGWLSRKIVKDFTAFADVCFREFGDRVLYWTTINEPNIFALGGYDNGQIPPGRCSFPFGKFCTEGNSSTEPYIAVHNMLLAHSSAVKLYRKKYKATQGGLLGINIYTFGVVPHTDSTADIIATQRTNDFYIGWIVNPLISGDYPDIMKKNVGTRLPVFAPAESKLVKGAFDFFGLNHYTSCFIEDDPNSLNRETRDVVADMAVQIQFPGSRFPPDQFPVIPSGLFSVLQYFKEVYGNPRIYVQENGQRTDRNTTLNDTPRIEYLQAYIGAVLDAIRNGSNTRGYFLWSFLDGFELLDGFKSSYGLYYVDLDDKELKRYPKLSAAWYSNFLKGRSNAMPDRLIDAANYISVS

SEQ ID NO: 13 - protein, 439 aa, Mitragyna speciosa
MADNSSGKVAIDSYHRHKSDVQLVKNLGLDVYRFSISWSQILPGGKLSKGVNQLGIDYYNALIDELVSNGIKPVVTLFHRDVPQVLEDLYGGFLSPRIVDDFRNYADVCFKYFGDRVKYWVTFNEPWSFSKEGYADGLSAPARCTYWYDSDCAGGDSGTEPYLVTHHLIIAHASAVRLYRQKYQSTQNGSIGITNVAEWYLPSTIGSARDEEAVRVQLDFKFGWFLHPITYGVYPKVMQQRVGNRLPRFTREQSKWLIGSIDFLGLNYYTGNFATFFDKSYIPKYPSYSTDSGVITTGFDSDGTDIGITAGSAWFRRYAVGLKELLNYIKTNYKNPPILITENGICTMGDTTEDSINDMYRVKYLEEHLCCLLRAIEDDKANVFGYIVRKMFDALESTQGYDDLSLKRITKTSTSYWLKNVLSTNDTSLSDHSRTSSGG

SEQ ID NO: 14 - protein, 353 aa, Mitragyna speciosa
MAGKCAQEEHTVKAFGWAAREASGALSPYGFSRRATGERDVKINVLYSGMCNFDTEMINNKFGFTKYPYVLGHETVGVVSEVGSKVRKFKVGDKVGVGGLVGSCRKCYSCTNDLENYCTKAELTEAGAGGCSNFVVTDEDFVFHWPEKLPLDLGAPLLCAGVTTFSPLKTHGLDKPGMHVGVAGLGGLGHVAVKFLKAFGAKVTVISTSDNKKREAIEKYGADAFLNSSNPEQMRAAAGTLAAIVDTIPSPHSLVPLLDLLLPHGKVIVLGAPSEPFVLPVMPLLQGGRVVAGSSGASLKQIQEMLDFAAEHNIVADAEVIPIDYINTAIKRIEKGDIKYRFVVDIGNTLKSA

SEQ ID NO: 15 - protein, 360 aa, Mitragyna speciosa
MAKTPEMVHPVRAFGWAARDTSGELSPFKFSRRATGEHDVQFKVLYCGICHSDLHMIKNEWGMTVYPIVPGHEIVGVVTEVGSKVEKVKVGDKVGVGCLVGSCGNCDMCSQDLENYCPKQILTYSAIDEDGSITYGGYSDVMVANEHFIIRWPENLPLDAGAPLLCAGITTYSPLRYFGLDKPGMHVGIVGLGGLGHVAVKFAKAFGAKVTVISTSENKKKEAIEKLGADAFLNSRDPQQMQAAVGTFDGILDTVSAVHPIVPLINLVKSQGKVIMVGAPEKPLELATFPLLVGRKTLAGSAIGGLKETQEMIDFAAKHNILAEVEVIPMNYVNTAMERLLKADVKYRFVIDIGNSLKSA

SEQ ID NO: 16 - protein, 363 aa, Mitragyna speciosa
MAGKSPEGQHPVKTYGWAARDSSGILSPFKFSRRATGDDDVRFKVLYCGICHTDLHAVRNDWGFSTYPLVPGHEIVGIATDVGSKVTKVKVGDKVAVGCFVGSCGKCENCTNDLESYCPGMITTYVGTYHDGTPTYGGYSNEMIASEHFIVRFPEKLPLAGGAPLLCAGITVYSPMKYYGFDKPGTHLGIVGLGGLGHVAVKFAKAFGAKVTVISTSPSKKDEAINHLGADAFLVSRDAEQMKASSGTFDGIIDTVAAVHPISPLIDLLKNHGKLILVGAPDKPLELPVFPLLMGRKTVASSGAGGLKETQEMVDFAAEHNIVADVEVIPMDYVNTAMERLHKGDVRYRFVIDVGNTLAPPGS

SEQ ID NO: 17 - protein, 362 aa, Mitragyna speciosa
MAAEKSPEDLHPVKCFGWAARDTSGILSPFKFSRRATGEKDVRFKVLYCGVCHSDLHCVKNEWGWTNYPLVPGHEMVGTVTEVGSKVTKCKVGDTVGMGCLCGSCRTCEQCKNDVETYCAELKMTYLSIYYDGTPTQGGYSNEMVADEHFIINWPENFPLAAGAPLLCAGATVYSPMKYYGLDKPGTHLGIVGLGGLGHVAVKFAKAFGLKVTVISTSPSKRDEAINQLGADDFLVSRDPDAMKAAMGTMDNIFDAVSAVHPLMPLFDLLKPHGKLVMVGAPTKPYEIVVPTLVMSRKMVGFAAAAGLKETQEMINFAAEHNITADIELVPMDYVNKAIERLAKNDVRYRFVLDIANTLKEE

SEQ ID NO: 18 - protein, 343 aa, Mitragyna speciosa
MAGENRSNVFGLAARKISLEIEISGENRVKTCGWAARDSSGVFSPFDFTRRATGEEDVRFKILYCGICHSDLHHAKDEFGFGIYPLVPGHEIVGIVTEVGSKVTKFKAGDKVGVGTIVGSCRSCNRCSNDLEPYCPKMMMTYNSIDEDGIPTRGGFSNEMVVNEHFAVRWPDNLPLDGGAPLLCAGSTVYSPMVYYGLSKPGTHLGVAGLGGLGHVAVKFAKAFGVEVTVISTSPSKKEEAINHLGADHFLVSTDQDQMQAAMGTLDGIIDTISAVHPIMPLFGLLKHDAKLIVVGAPNKPLEVDIPVLIIGRKMLGASAVGGMKETQEMIEFAAKHNITADI

SEQ ID NO: 19 - protein, 361 aa, Mitragyna speciosa
MAQTTPNHTQSVSGWAAHDSSGKITPYVFKRRENGINDVTIEVLYCGMCHTDIHHVKNDWGITMYPVVPGHEITGIITKVGSNVTKFKIGDKVGVGCLAATCLECEFCKDSQENYCDQVQFTYNGIFWDGSITYGGYSKMLVADHRYVVQVPDSLPMDAAAPLLCAGITVYCPLKDHNLLEPGVAAKKIGVVGLGGLGHVAVKFAKAFGHHVTVISTSPSKEKEAKERLGADDFIISTDMKQMQAKKRTLDFIVNTVSAKHSLGLLLELLKVKGTLVIVGAPDKPLDLPSFPLIFGKRVVKGGIIGSIKETQEMMDLCGKRNITCDIELVQTDQINEALERLAKNDVKYRFVIDIAGKSST

SEQ ID NO: 20 - protein, 357 aa, Mitragyna speciosa
MGSLDVERKTVGWAARDPSGVLSPYTYPLRNTGPEDVYIKVICCGICHTDIHQVKNDLGMSNYPMVPGHEVVGEVVEVGSDVTKFRVGECVGVGAIVGCCGNCRPCTADIEQYCNKKIWSYNDVYTDGKPTQGGFAGAMVVDQKFVVKIPDGLSPEQAAPLLCAGVTVYSPLNHFGLKESGLRGAIVGLGGVGHMGVKIAKAMGHHVTVISSSDKKRGEAIDHLGADDYLVSSDTTRMQQAADSLDYIIDTVPVFHPLEPYLSLLKVDGKLILMGVINTPLQFVTPMVMLGRKTITGSFIGSMKETEEMLEFCKEKNLASMIEVVKMDYVNTALERLEKNDVRYRFVVDVAGSKLEQ

SEQ ID NO: 21 - protein, 355 aa, Mitragyna speciosa
MTSASDKEDCLGWAARDPSGFLSPYKFSRRAIGSEDVSLDIAYCGICYADVAWTRNKMGHSKYPLVPGHEITGVVRQVGSQVKRFKIGDRVGVGTYVNSCRECEYCDEGLEVHCSKGQVFTFDSIDVDGTVTKGGYSSYIVVHERYCYRIPDNYPLELAAPLLCAGISVYTPMMRYNMNQPGKSLGVIGLGGLGHLAVKFGKAFGLKVTVFSTSISKKEEAVNLLGADNFVVSSDEQQMSALAKSLDFIINTASGDIPFDVYLSLLKTAGVLVLVGFPSEVKFSPVNLILGMKIVTGSVTGGTKQTQEMLDFCASHKIYPEIEIVPIQYSNEALERMIKKEVKYRFVIDIAHSLK

SEQ ID NO: 22 - protein, 309 aa, Mitragyna speciosa
MKSNQIYFEFVVAFSFGLCRHEMVGTVTEVGSKVTKFAVGDTVGVGCLVGSCGSCDDCCNDLENYCPNMILTYLSKYHDGTPTQGGYSNEMVADEHFVIRIPENISLDACAPLLCAGITVYSPMKYYGLAKPGVHIGIVGLGGLGHVAVKFAKAFGAKVTVISTSPSKKEEAINQLGADSFLVSRDPEQMKAATGTMDGILDTVSAVHPIMPLIDLLKSSGRLLMVGAPDKPLELLVFPLLLGRKGVSGSSIGGIKETQEMIDFAAKHNITAEIELIPMDYVNTAMERLAKNDVRYRFVIDIANTLVVP

SEQ ID NO: 23 - protein, 506 aa, Mitragyna speciosa
MEYIFLLCALLFSLMLTKIVIKSKNNNSWKKLPPGPRQVPIIGNMHQLYGPLPHHKLRDLAKKYGPLMHLQLGEISTIVVSSPEFAREVYRTHDIIFAERAELLSISIVSYNFLGIVFAPYADYWRQLRKICTMELLSPKRVQTFRSIREEEVLNMIKSIALQKGSSVNLSRKIFSLTYGITAQAAFGQKGKYQEQFIMLVDEMVKLAGGFSLVDMYPSIKLLERISGTRTKLEKLHKQIDGILQTIVNEHKKKLEKEELGSGEKKVDLVDVLLNIQKRGEFEPPLADTNVKAIIYDIFSAGSETSSTTVEWAISEMIKSPAVMKRAQDEVRNIFKERRNVDESNLDELKYLQAVIKETMRLHPSAPLLLPKESTEKCEIKGYEIPAKTRVIVNAWALGRDPMYWSEAEKFNPERFIDSELDFRGNHFEYIPFGAGRRICPGISFALPNIELPLAQLLFHFDWKLPGDLKQEQLDMTEVFGVTVRRKNDLQVIPVPYSHSSLNKDL

SEQ ID NO: 24 - protein, 506 aa, Mitragyna speciosa
MELFTILCAFFLFLFMLVKFLNPDRVKVPAQTLPPGPTPLPIIGNLHQLLGSNTHHILKELASQYGPLMHLQLGQVSTLIVTSPEVAEEFMKTRDIIFANRPQLFAGRILRYNCTNIGFSPFNDYWRQLRKICTMELLSSKRVQSFQSIREEEVLNLVESISSNWGSTINLSRRICSLAYGITARAAFGKRSKYQEEFISLIEEVVKIAAGFTIADMYPSVKIIQIISEMSPKIKRLHKNIDAILENIVDDHKEKNTKTRGTDEEAKDDLVDVLLNVQKSGEFGAPLTNNNIKAVILDIFSAGSESVSTTVEWTMSEMLKNPDIMKRAQAEVREVFGRRRNVDESSLHELKYLQAIIRETLRLHPPGPLLVPRESSEQCEVNGYIVPVKSRVIVNAWAIGRDSKYWTEAEKFIPERFLDSQVDYHGKDFKYIPFGAGRRICPGISYALANVELPLAQLLFHFDWKLPNELKLEQLDMTEAGFALTVRRKNDLYLDPIPYSRSIFSN

SEQ ID NO: 25 - protein, 398 aa, Mitragyna speciosa
PIIGNMHQLHGSPIHHLLRDLAKKYGPLMHLKLGEISAIIVTSPEMAKEIYKTNDLLFASRPSPHLAFKIISYNFVDIIFSAYGNHWRQLRKICTAELLSPKRVQTFKSIREDEVFNLIQSISSQKGSIINLSRCIFPLSYSITSRIAFGKRNKYTERFIQLVEEINKLVSGFSLADMYPSVKLLQVMSIMRYKLEIAHRQVDQILENILNDHKQKITDAKQEGGERKEDLVDVLLSIQEGGDSEPELTDTAIKAVIFDIFSAGSETSSTAIEWALSELIRNPEVIKRAQDEVRNVHDERGNVDESSLHELKYLHAIIKETLRLHPSAPLLLPRECGEQCEINGYVIPAKARILVNAWAIGRDPMYWTEAEKFNPERFLDSEIDFKGNNFEYIPFGAG

SEQ ID NO: 26 - protein, 500 aa, Mitragyna speciosa
MELFLTLCALLAFFSIALKIVRKTKLVKLPPGPRPLPIIGNLHQLNGSLPHRILTDLAKKYGPLMHLQLGEVSTVIVSSPAVAKEVMKDHDIIFCYRPLLLSPAILNYGGTDIAFAPYGEYWRQLRKICTIELLSSKRVQTFRSIREQEVSNLFRSIKSAEGSVVNLSKMIYSLTYSITAQAAFGKESKYQDKFISVMQDAIKLMGGFNIADVYPSIKILEKITGIRHKLEETHNQIDEIVQNILIEHKAKRAESKLGNRGAKEDLVDVLLNIQSSGEFEPPLTDDNLKAVIYDIFSAGGETSSTTVIWAMSEMIRNPKVMKKAQDEVREVFAGNGNVDESRLHELKYLQAVIKETMRLNPAVPLLLPRECSEHCQINGYDVPAKTRVIVNAWAIGRDPKQWTEPEKFKPDRFLDSEIDFRGKTFSFIPFGAGRRICPGISFALPLVELPLAQLLYHFDWKLPGQSKPDELDMTEIFGLTVGRKHDLNLVPIPYRPCSVL

SEQ ID NO: 27 - protein, 442 aa, Mitragyna speciosa
MNHLEIYICYCYHLLSSIFSPHGGHPLFCAIIFLFLALKLLKRSTKKSALHLPPGPKPLPIIGNMHQLFGSLIHRILRDMAETYGPLMHLRLGEVSTLVVTSPEVAQELLKTHDIIFANRPQLLCPRMFNYGCTDIAFSPYGEFWRQLRKICVTELLSPKRVQSFRPVREEEVLKFIRMVFSKEGSTVNLSRMLFSFMYGLTAQVAFGKKNKNQEEFISHIEEATKMTSGFNIADVYPSVKFIQVLSEMSPKMKKMQKNIDKILENIVDEHTNKNQQTEPTDGELKEDLVDVLLNIQKSGDLKIPLNRNNVKSVIMDVFTAGSETSSTVLEWAMSELIRNPGVMKKAQEEVRNAFDGSGNVCESGLPELKYLQAVIKETLRLRPPVPLLIPRESSEQCKINEFDIPARTRVMVNVWAINRDHRYWIEAEKFDPERFLNCTID

SEQ ID NO: 28 - protein, 508 aa, Mitragyna speciosa
MTYFHFNFITLFIFVAFIMSLVKKWKRSEQLKKLPPGPWKLPVIGNIHHLIGPPPHHILKNLAHKHGALMHLQLGEISAIVISSPRLAEEIMKTHDLAFANRPELLVSKILCYNSSDIVFSPYGDYWRQLRKICTLELLSAKNVRSFGSIRQDEAFHLISSIRSLAANGTPINLTKTISSFTSSIICRAAFGKVCRDDQDKFIQIMKDSIALTGGFDISDLFPSWKILHGLSRMKPKLLMVQHEFDTILDSIINQHIENLEKTRNDGDPGDEDLIDVLLRVKKSGDLQFPLTKSNIKAVVYDMFTGGTETSSTTVEWAMAEMIRNPNVMAKAQNEVRKAFMAKKTIEESDIQELRYLKLVIKETLRLHPPVPLLVPRECREECEIDGYVIPVKTRALINAWAIGRDPEYWSDPDIFQPERFEQNSCEFTGVNFKYLPFGAGRRICPGLQFGLANTELPLALLLYHFDWKLPDSMNSCCLDMTETCGMTAARKNNLILAATSYDPHDTS

SEQ ID NO: 29 - protein, 453 aa, Mitragyna speciosa
VELQNCPSNFISFFLFAAILLTIIKEWRTSKKLKTIQKLPPGPWNLPFVGCMHHLIGGLPHHSLKNLAQKHGPLMHLQLGEVSAIVVSSPNVAKEIMKTHDISFASRPELLALKNMFYGSIHIAFSPYGDYWRQMRKIRILELLGAKNVRSFGNIWQDEVLHLVEAVRNLACKKVNLTEQIFSYASSMVCRAAFGQVSKDDKSEFAQLMKQVAALTGGFDIADLFPSYKILHVLSGMKPKLSKVHQKIDVMFENLIKEHDENRNRRNKGGAEFGQEHLIDVLLRIRDSGDLQIPITNNNIKAIIFDMFAAGTETSSSTVEWAMSEMIRNPNVMAKAQNEIRQAFMGKQKIDEADIQGLRYLKLVIKETLRLHPPFPLLLPRECREQCELNGYTIPVKTKVMVNAWAIGRDPEYWRDPEIFEPERLEHNLVDFTGNHFEFLPFGAGRRICPGMT

SEQ ID NO: 30 - protein, 514 aa, Mitragyna speciosa
ASFQMEMHLSFFTLTALFLLLSFLFLLIKEIKGQKNTRDAKKLPPGPKQLPFIGNLHQMVGSLPHHKLRKLADKYGPIMQLQLGELSTIVISSTELAKEVLQTHSAAFANRPQLMVAKIMLYNSLGVTFSPYGDYWRKMRHMYITELLNTKSVHSLFGILEDEVSKLTMSIESLAGKPIILGEMILSYLNTAISRATVGRICKDQDALIMATREAASLAGIFNLADLFPSVKILQLVNRSKAKLEETYRKLDGILEDIISGHEKNKIGTKADNQNPAEEDIVDILLRLKKSNDFQLPITSSNIKAIIFELAVAGTITSLVAIEWAISELMKNPKVMEKAQAEVRQAFKGQKKISGVDIQKLKYLKWVIKETLRLHPPGPLLAPRECREQCEISGYTIPINTVTIINAGAIGRDPKYWNNPENFEPERFSNSSIDFTGNSFELLPFGAGKRLCPGINYAVANIEILLANLLYHFDWKLPGGITPEEFDMTEKFAAAVTRKDDLCLLAKSYVPSDV

SEQ ID NO: 31 - protein, 507 aa, Mitragyna speciosa
MELRFIPFSLSSINLFLLLSFLFLLVKLWKNFKTSNIAQKLPPGPPKLPLIGNIHNLIGGLPHHVFRDLAKIYGPLMHLQIGEVLTVVLSSAKLAKDVLVTHHPSFASRPSNLAIKIIWYDQEGMGFTSYGEHWNQMRKICMLELLSIKSVASFKPIRQDEISKLVGSIQSTLGVPVNLTEKIFAYTSSVICRAAFGRVCKDKEKMIKNLKIALALAGGFNLADVFPSLRLLPIITGFKQKLIKIHHEMDEILCDVVKEHIANHESGKKGNAETGDQDLIDVLLLQQKTSIQIPITVQNIKAVIIDIFTAGTDALSDTTEWAMAELMRHPRVMAKAQEEVRQLFKGKKTIEEADVQKLKYLKMVIQETLRLHPPAPLIPRASRENREVNGYMIPDKVQVLVNVWAIGRDPEYWDDPEEFIPERFEQKSVDYLGTQSEYIPFGSGRRMCPGATFGLASVELSLANLLYHFDWKLPNGMEPCDLDMDETAGVTAGRKNSLYLVAIACDP

SEQ ID NO: 32 - protein, 260 aa, Mitragyna speciosa
MFIVCNIRSDSDMEIELLALFLTFFSMLLLLLFGSRFRTNNSISHLPPGPWKLPLIGNIHQIVGSPPNRALRDLAKKYGPVMQLQLGEVSTIVVSSAETAKEVMRTHDIIFASRPHIIATKILSYDSTNIGFSPYGEYWRQLRKICVSELLGASRVQSFRYIREEETLDLIRWKACNAGSMINLTQKIRSFTYATISRAAFGKKSAEQETFINTVTDCAKLAGGFNIADLYPSVKFLDVISGLKTKLRRLHRQDTWEHHQ

SEQ ID NO: 33 - protein, 307 aa, Mitragyna speciosa
MELIPLPTSFITSILLLFLFLKLLPKFTTSSKKVGSPKLPPGPWKLPIIGSMHHLAGSLPHRALAGLAKKHGQIMHLQLGEISTVVISGARMAKEVLKTHDVALANRPKFLAAEIITYNYQDVAMAPYGDYWRQMRKICVLELLSAKNIRASRFIREDEVWKMVHSIQSSSSSMSRKVYLSEKVTALTNAVTCRASFGSRCKYQDELVKLINEIMEVSTGFDIADLFPTKKFLQIISGTISRLKKLQSKLDPIFEDIIQEHKEMNPAARGQSEDPENLVDVLLKVNERGGLDFPISTSSIKAIFVVS

SEQ ID NO: 34 - protein, 511 aa, Mitragyna speciosa
MALFEWEKEGFPSPYLLIFASVSLIVVLKFVSKPKNNRNSKLPPCPPKLPIIGNLHLLGNMPQESLHQLAKKYGPVIFLQLGEVPTIVISSARLAKEAMKTFDLALSSRPQIFSAKHLFYNCTDVVFSPYGAYWRNIRKICILELLSAKRVQSFSYVREEEVAHLVQRVAEAYPGTTNLTKMLGLYANNLVCRVAFGKDFSQGGDNHRHNFQKLLEEYQVLLGGFSIGDFFPSMEFVHKFTGMESRLKDTFRRFDQFFDEILQEHRNPESRKEHKDLVDVLLEIQKNGDPETPLTTDNIKSIILDMFAAGTDTNFITLDWAMTELMTNPGVLKRAQAEVRNIVGERRSVSENDLPQLPYVKAVVKETFRLHPPAPVLVPRESMEDVTIDGYDIPAKTRFFINAWAIGRDPKSWENPDVFEPERFMNSHIDFKGQDYELIPFGAGRRSCPAITFSAVTVELALAQLLHSFDWELPPGVEAKDLDMTEVFGITMHKIYPLMVVAKPYFSQGLN

SEQ ID NO: 35 - protein, 533 aa, Mitragyna speciosa
MERGKIQGKLRSMASSSGLVSDLKFEESILHPIFFSLFPLIILLFLFKFLSNTRKNQPPSPPGFPIIGNLHQLSSLPHYPLHSLAKRYGPIMLLKFGSVPTVVISSADAASLIMKTHDLIFSDRPFSRTANKLLYNMKDISIAPYGEYWRQLKSICVLQLLSHKKVQAFRNIREEETSVMMDKIKEASLNLTPVNLSEMLFSLTNDIVCRSAFGRKYGEGESGKKFKLLLSEFLKLLNTPSLADFVPWLGWVNRVNGFDASIDRVAREIDEFLESVLHERLVATLGNDSRSSDETIVCESKEDFLDILLNIYKENAAGVTMDRESVKAIILDVFSAGTDTTATVAEWAMTEILRHPIVKERLQNEIKGVVGSNRDITEYDLEKMPYLKAVIKETLRLHPPIPLLVPRKAREDVRIMGYDIAAGTMVIINAWAIGRDPAFWEEPEKFKPQRFLDSSIDFKGHDFQLIPFGAGRRGCPGIAFAIASNELVLANLVRKFDWRFPDGTKGEELDMTECPGVAVHRKIPLLAIPTPLS

SEQ ID NO: 36 - protein, 573 aa, Mitragyna speciosa
MAEVIFSSFLTTFCSFSTITIIFSPFLTSTKTRIFSISHTFDLHIEQDIHQKQNKMDNFTPEILCTIFLSFAAFCFYYYYIIHRRTRSPPVTLPPSPSKLPIIGHLHLLTDMPHLRFSQLAQKLGPIIYLQLGQVPTVVISSAKLAELVLKTHDHVMANRPQIIAAQYLSFGCSDVTFSPYGPYWRQARKVCVTELLSSKRVNSFRLIRDEEVNRMLSTVSAHANSELDVSELFFQLANDILCRVAFGKRFMDENNEETGKKNELVGVLTETQALLAGFCIGDFFPSWKWVSSVSGTKRRLMNNLKDLRMVCDEIINEHVRRREHRGPSADVLDKEDFVDVLLRVQKQDDLEVPITDDNLKALVLDMFVAGTDTTSATLEWTMTELARHPKIMKRAQDEVRQIAASKGKVEESDLQHLHYMKAVIKETMRLHPPVPLLVPRESMAKCTIDKYEIPANTRVLINTYAIGRDAESWEDPLEYNPERFLGKDIDFKGQDFRFLPFGGGRRGCPGFSFGLASVEISLARLLYRFDWALPEGVGANDVDLTEIFGLATRKRSALKLIPTFNNQHARVI

SEQ ID NO: 37 - protein, 514 aa, Mitragyna speciosa
MAKQIFVLDLPFSSLFPLALLLLTLVIWFYASSRPQKRLPPSPPKLPIVGHLFRLGIYPHRTLQRLSKKYGPLMMIHLGSKPILVASSADVACEIMKNHDLVFANRPKRSINSKLLYDCKDIATAQYGEYWRQIRSICVLQLLSNKRVQSFRHVREEETSMMIQKIRERCSSSSSSLINLSDALITLTNDVICRVALGRKYSNDENGRKSMKIMKEFGELLGTFSVGDYLPWLAWVNRFNGLDAKLEKVAKHIDQFLEGVIEEHKFRKKGEDYVDSTEKKALDLVDILLDIQKDNSVGLALELDSVKAIILDMFAGGTDTSYTAMEWAMSELLRDPKTLEKLQVEVRKVAQGKSEITEDDLDKMHYLKAVIKETLRLHTPIPLLVPRESTQHVKILGYDIPAGTEVMVNAWAIARDPVQWKKPEEFLPERFLNSTIDFRGFNFEFIPFGAGRRGCPGTTFAIAVNELALAKLLHEFDFALPDGAKPEDLDMSDATGFTVHRKFPLLAVAIPHSC

SEQ ID NO: 38 - protein, 501 aa, Mitragyna speciosa
MGTLIVLFSILPIVILIILQNASKKPSKKIHPPPPGPPGLPLIGNLHQFDSSTPHRYLWQLSRKYGPLMSLKLGSVPVLVVSSAKMAEEVMKNHDLIFCSRPPMHGQRKLSYNGLDIAFARYGEEWREMRKVAVLHLFSNRRVQSFRSIHEDEVYRMTQKISTESASSQVTNLSRTVLSLTSTMICRIAFGKRYDEKSLERIRFYDLLHEVQSAFVGFYFSDYFPSLGWVDYCTGMLSRLEKTFNNLDLFYEELIEEHLHPNRPKSMQGDIIDLMLHLRNDKSTPFDLTMDHIKAMLMDMFTAGTDTVGAAIIWAMTALIKSPRAMKKAQAEIREVIGNKKVVGEDAAQKLPYLKAIIKETFRLYPPAPLLVPRQTMENCVIDGYEIKAKTIVYINAWAIARDPKYWENPDEFLPERFLNSTVDLKGQDFQVIPFGAGRRGCPGYSLGLATVELALANLLYSFDWELPCGMRKEDIDVDVLPGLTMLKKNDLQLVAKNVEV

SEQ ID NO: 39 - protein, 370 aa, Mitragyna speciosa
MLLQLGSVPTLVVSSADMAREIFKRHDPAFSGRPVLYVAKKLSFNCSALAFAPYGEYWRQVRRILVLQLLSTKRVQSFEAIRADEVALMVKFIARCSNNNPVNLSKLAFKLANNIICRVAFGRSDDGNAKFREILYETQALLGESNIADFFPRMAWFNKFNGIESRLEKNFRELDGFFNEVIKVHLDPGKFKPEHEDLVDVLLRSPRDPTQTISLSNDDIKGVLTDILVAGSDTSAATIEWTMAELIRNPTAKRKAQQEVREVMKAKGKVEESDLSRLKYLKLVMKESLRLHPPAPLLVPRETLESCKIGGYQIPAKTRVLINAASIATDPTCWENPLEFKPERFLNSSVDFRGQNFELLPFGAGRRSCP

SEQ ID NO: 40 - protein, 512 aa, Mitragyna speciosa
MSTLTFIFITSLLAFLLYSLLKKILNPTKPLPPGPKPWPILGNLPHLGTKPHHSLAAIAKTYGPLMHLRLGFVHVVVAASASVAAQFLKTHDANFSSRPPNSGAKHIAYNYQDLVFAPYGPRWRMLRKICSVHLFSAKALDDFHLVRQGEVSILTRALASAGNNPVNLGQLLNVCTTNALGRVMLGRRVFGDGSGGGDPKADEFKSMVVELMVLAGVFNLGDFIPVLDWLDLQGVAAKMKKLHARFDAFLNTILEEHKINGSDGDKGHVDLLSTLISLKDNADGEGGTLSDTEIKALLLDLFTAGTDTSSSTVEWAIAELIRHPKLLAQAQQELDTVVGPNRLVTEADLPQLTYLQAIIKETFRLHPSTPLSLPRIAAESCEINGYFIPKGSTLLVNVWAIARDPDMWTDPLEFKPQRFLPGGEKHNVDVRGNDFEVIPFGAGRRICAGMSLGLRMVQLLTATLVHAFDWDLPNGQTAEKLNMEEAYGLTLQRASPLMVHPRPRLAPHAYRT

SEQ ID NO: 41 - protein, 524 aa, Mitragyna speciosa
MVYLIWNYILFQSVDQESKNHHPKVMMPSAWIWPAFTLLAIVSFLNSLLRKNKKKKLPPSPRGLPILGHLHLLGKNPHQDLHKLSKQHGPIMHLRFGFVSNIIVSSPHAAEQFLKTHDLVFASRPPHEAAKYIDFGQRNLSFGQYGSYWRNMRKLCTLNLLSQLKINSFQSMRREELGLFLKSLKEAALNRDVVDISAEVAALNANMSCLMVFGKKYADNEFDKRGFKAVIKEGMQLSATPNLGDYYPYLGVLDLQGLTRRMKAIGKVFDEFFEKIIDEHEQSENQARQADDFVYTMMALMKSGETEFQFDRRHIKAILLDMLAGSMDTSATVVEWILAELLKHPRVMKKVQRELEEVVGLNRMVEESDLDSLKYLEMVVKEALRLHPVAPLLIPHASMEDCTVDGFYIPKNSRVIINVWTIGRDPNAWSDPEEFIPERFVGSNIDLSGHDFQLLPFGSGRRGCPGMQLGLTVVRLLVAQLVHCFNWELPNGMSPKELDMTEEFGLVVTRAKHLMAIPAYRLSK

SEQ ID NO: 42 - protein, 404 aa, Mitragyna speciosa
MEFQFISFPLNFLNLLLLFGFLILLVKIWQKQNTSKIRLPPGPLKLPLVGNMHNLVGGLPHVVLRDLAGKYGPLIHLQLGEVSMVVVSSPEMAKEVLVNHDPAFADKPECLATKIMWYDQQGLIFTPYGDHWRQMRRICMTELLSAKIVRSFSFIRNDEITKLMESIRSSLGFPINATELFFNFASSMTCRAAFGGICKDNETLIAYLKEGAILASGFNVADAFPSLKILPIISRLKGKLLEMHHKTDLILDDLINQHKVNHEKGKKGNAESGDQDLVDVLLRQQENGNLQIPITSRKIKALLFDIFTAGTDTSSITTEWAMSELMKHPSVMAKAQAEVRQVCNGKKTIEEADIQKLVYLKMVVKETLRLHPPIPLIPRASNENGEVKGYMIPDKFQVMVNAWA

SEQ ID NO: 43 - protein, 373 aa, Mitragyna speciosa
MDFTFNFIAFFLSLAFVLTLCKKWKRYKAAEKLPPSPWKLPIIGNMHHLIGSIPHHAFRKLSQKHGPLLHLQLGEISSIIVSSPRLAKEVMKTHDLAFASRAEFLGTKIVRYNCSDIVSSPYGEYWRQMRKICTLEIFSAKSVRSFGSIRKDEAMHLIAAIHDLAAAQEPINLAEKLFSYTSSVLCRVAFGKLSKNQQSAFVQLNNESVLLFSAFDISDLFPSLKILHPFLSMKTKLVKIHHKMDLLLENIIDQHIDNLARTKMATGESGIKDLIDVLLRVKENGDLQIPITKNNIKAVVLDIFSGGTETSSGTVEWAMSEMIRNPTVMAKAQSEIRKAFTGKKTIEETDIQDLRYLKLVIKETLRLHPPVPL

SEQ ID NO: 44 - protein, 513 aa, Mitragyna speciosa
MAEVEGYIHLFLIWLIPTILLQILFRKRTVSRLPPSPLALPIIGHLHLLAPIPHQALHKLSNRYGPLIHLYLGSVPCVVASSPEMAKEFLKTHENSFSNRPKSAVIDYITYSSQDFSFAPYGPYWKFMKKLCMSELLGGRTLDLLLPVRRDEIKRFMELLERKAKATEAVDIGAELIRLANNVVSRMAMSKRCSENEDEAGDVKKLIHEIAELTGMFNLSDFIWFCKNLDLQGFKKRIKDVAERFDAMIEKIIEEHQKTRRMHKQSNDAGQEAKDLLDILLDVSEDESSDIRLTRENIKAFILDIFAAGTDTSAITVEWALSELMNHPNIMQKAVQEIDSIIGKNRLVDELDIKNLPYLQAVVKETLRLHPTGPIIVRESSEDCEIGSYHIPAKTRLFVNVWAIGRDPKSWENPLEFRPERFLFEEGSENKSTLDVRGQHFHFLPFGSGRRGCPGTSLALQVVQTSLAAMLQCFEWKINGKVDMEEGPGLTLPKANPLVCTPVARLNPLPIPK

SEQ ID NO: 45 - protein, 511 aa, Mitragyna speciosa
MDSFPSNWAAYALVWLATVVIVLLSKHFRKKKLNPPPGPKPWPIIGNLNLIGSLPHRSLHQLSLTYGPLMQLRFGSFPVVVGSSVEMAKVFLKTMDVTFAGRPKTAAGKYTTYNYSDITWSPYGPYWRQARKMCLTELFSAKRLESYEYIRVEEMNSLILGLFKSSGKPVLLKDYLSTVSLNVISRMVLGKRYLDESENSIVAPEEFKKMLDELFLLNGVFNIGDSIPWLDFLDLQGYIKRMKILSKKFDRFLEHVLDEHIVRRKDEKNCASKDMVDVLLDLADDPTLEVKLERHGVKAFTQDLLAGGTESSAVTVEWAISELLKNPELFEKATEELDRVIGQNRWVKEKDMPNLPYIEAIVKETMRLHPVAPMLVPRCSREDCKVAGYDIQKGTRVLVNVWTIGRDPQLWEKPAEFHPDRFIGKDIDVKGQDYELLPFGSGRRMCPGYSLGLKVIQSNLANLLHGYKWKLPNDMKPADLDMEEIFGLSTPRKIPLVACVEPRLPRHLYSL

SEQ ID NO: 46 - protein, 275 aa, Mitragyna speciosa
MEFFFLVCVIIFCFMAVKVVKKSRGKSLQRLPPGPTQLPIIGNIHQLRGSLPHRTLRDLAEKYGPLMHLQLGELSMIIVSSPQVAEEIFKTHDVIFSQRSNLIASSIINYYLVNIIFAPYGNYWRQIRKICTMELLSPTRVQTFRSIREEEVLNMMKSISVKEGSVLNLSKMIYSLTYGITARAAFGKPRQDQEEFKALIEKITEAFGGFSIVDMYPSVKLLQVISGMRFKLKKIHNRVDDIIQNILNEHKEKTSKQEPGSGETKDDLVDVLLNI

SEQ ID NO: 47 - protein, 433 aa, Mitragyna speciosa
MVLLFLIILLVLIILTHQKNKKVGKRCHPPGPPGLPFIGNLHQFDAEKPHKFLWRLSKKYGPIMSLQLGFVHVVVISSARIAEEALTTHDLVFSGRPAAVGRRKLSYDRRDIAFSPYSEYWRDMRKICVLHLFSLKRVESFRPIREYETSYMIQKIAKHSSLSQPINLRVLIMSLTSTIICRLAFGKRYDEEGHERKRFDELLLESQAMIAGFFVADYLPSLSWLDKLFGMMTRLEKNFNELDLFYKELIEEHLNPNRPDTMKNDLLDLLIQLKQEQSSTVGFSWEHIKAILMDIFVAGTDTSAATIIWAMTALMRSPSAMRRVQVEVREVVGKKGAVDEEDIHELPYLKAVIKETLRLYPPAPILGPRETTERCNLHGYPIESKTLVIFNAWAIARDPECWKNPDDFFPERFLNSNIDVKGHDFEVIPFGAG

SEQ ID NO: 48 - protein, 517 aa, Mitragyna speciosa
MVKKMGSLVEALDTETMMLFFIVPLVFLFLVSRFRRKPHPPGPKGWPLIGNMMIMNQLSHRGLAQLADQYGGLFRLKMGFLNMVAVSSPEIARQVLQVQDNIFSNRPATIAISYLTYDRADMAFAHYGPFWRQMRKLCVMKLFSRRRAESWDSVRDEVDDMIKITASNTGSAVNLGELVFGLTRNIIYRAAFGTSCREGQDEFIQILQEFSRLFGAFNLADFIPWLNWLDPQGLNKRLVKARASLDGFIDSIIDDHMEKKKKMSGSVVEGDSDMVDELLAFYSDEAKVSESEDLQNAIRLTRDNIKAIIMDVMFGGTETVASAIEWAMAELMKSPEDLKKVQQELSDVVGLHRKVEESDFDKLTYYKCCLKEVLRLHPPIPLLLHETAEDSEVAGYYIPAKSRVMINAWAIGRDKDSWEDANMFKPSRFLKDGVPDYKGSNFEFIPFGSGRRSCPGMQLGLYALEVAVAHLLHCFTWDLPDGMKPSELDMDDIFGLTAPKASRLVAVPTPRLLCPLY

SEQ ID NO: 49 - protein, 508 aa, Mitragyna speciosa
MENTWLFLALASLVALAFLSKVSSDRRSKLNHPPGPKPWPIVGNLNLLGSIPHQSLHSLSQKYGEIMQLKFGSKPVVVASSPEMAKEFLKTHDHIFASRPTTAAGKYTSYNCSDMTWAPYGPYWRQARKIYLTEIFSPKRLDFFKSIRVEERNTFISNLFALSGKPVVMRDHLMRLGQSTSCRMVLSNKYVAQSERDGSLVTFEEFQEMIDTWFLLGGVFNIGDWISWLDRFDLQGYVKQMKELNKKFDRFHNQVIDDHLAKRKTERDFIPKDMVDILLQLAEDPNLEVKLTSDHIKGLIQDLLAGGIDTSATTVEWAMNELLKQPSLIGKATEELDRVIGRDRWVEEDDFSKLPFIEAIIKETLRLHPLATLLAPRYAIKDCTVAGYQIANGTTVFINTWSIGRNSRYWDSPEEFLPERFLEKDVDMKGQNFALLPFGSGRRRCPGYNLGLKLVRSMLANLLHGFNWRLPHGMAPEDICMEELYGLTTHPRISLALIPEPRLNVNLY

SEQ ID NO: 50 - protein, 523 aa, Mitragyna speciosa
MSSFQASQEEAKRWLLNDSGVVSLLLPWFVIFSLFISTWWFLTTSKKKNPPPSPPRLPIIGNLHQISSLAHRSMKSLADKHGPLMLLHLGSQPVLVATTADATREVLKTHDVAFSGRPESAVTQSIFRNVKNISLSPYGDSWKHVRSMAVNLFLNQKKVQSFRSIREEEVSLLVERIKESCASSSVICMNILLTTFANDTVSRITVGKRYSGQDGLKLAEILTTGAELLGAYMIWDFFPRLAWIAYLIGLEAKIKKVAKDFDQCLDNLVEEEMNRNKTGGSDSDVGEGDQGNDNQNLLQALVELHRTNSTGYPLDRKIIKGLVVDMIAGGLDIYSLLEWAMAMLIKHPDVMKKLQDEVKEFAGSKSFVSEGDLSKLQYLKAVIKETFRFCAPGAFIPRIATKDVKVMGYDIAAGTQLLVNKWALGRDPTLWEKPEEFRPERFLDSSIDLKGQNFELLPFGSGRRVCPGTTFALLIVELAIANLVCNFNFALPDGERAEDLDITEAPGVMSRRKTPLLLVPSLR

SEQ ID NO: 51 - protein, 523 aa, Mitragyna speciosa
MLQIFANTFYNGSKFTNDQLLLVIFSYVLCGLALIWFVVMYVKKSNKGQPPLPPGPTALPLVGNLLSLDPQLHVYFTTLSRTYGPILRLWLGKKVAIVIGSPVLAREVLKDQDITFANRDVPASAREATYGGSDIAWTPYGPEWRMLRKVCVREMLSNATLDSVYSFRRRELRQTINFMYSQAGKPVNVGEQMFLTVLNVITNMLWGGTVKGEERASLGAEFRQVVNEMTQCLGMINVSDLYPGLARFDLQGVQKKTKVLAGRFDRIFERMIDKRAKGIADEDDKESKDFLQFLLKLKDEGDSKTPLTMNHIKALLMDMVVGGTDTTANTVEFALAEMMNKPEILKKVQQELETVVGKDRIVEESDIQKLPYLDAVMKEVLRLHPALPLLIPHCPIETCIVGGYTIPKGARVFLNVWAIHRDPSIWENPTEFRPERFLNSKWDYSGNDFNYFPFGSGRRICAGTAMAERMFMFSLASLVHSFDWKVPEGEKLDLEEKFGIVLKMRVPLVAIPTPKLSDASLYE

SEQ ID NO: 52 - protein, 511 aa, Mitragyna speciosa
MELAQLQFVWGMTLLIPPLLILLLRRKKSSFNRLPPGPPGWPIFGNMFDLGSMPHKNLAGLKQKYGPIIWLRIGATNTMVVQSSKTAAELFKNHDIYFVERTVTEAMKSHGFDKGSLSLAPYGSYWRVMKRIMTVEMSVNKRINETVAIRRKCIDDMVSWIEKEADARKESRRGIHLARFVFLASFNMLGNLMLSRDLVDPESEEGMEFFSAMVGLMEWVGHPNIVDLFPWLRRLDPQGLRRKAERDMRKTMQIVSKFVKERLQDRQTGGNRKKDFLEVLLEFEGNGKDEPAKISEHDLNIIIMEVFIAGSETTSGTTEWAMVELLSNPTTMSKLKNELNEVVGRGKKFQEGDIDNLKYLQAVVKETLRLHPPIPLLVPRRATQDTNFMGYDIPRDTQVFVNVSAIGRDPECWEDPNSFKPERFLNSNIDFKGNHFELIPFGAGRRICAGIPLAYRMLHLVLGSLVHEFDWYVHNSVSDDVRDTKERMGVVVRKTEPLIAMPISKNSANKG

SEQ ID NO: 53 - protein, 501 aa, Mitragyna speciosa
MENMALLLDIGEYFLLLPIFFLPLLYFIFKQFKQSFASKTPPLPPGPTPWPVLGNIPHMGKMPHVTLSNFAETYGPLMSLKLGTQYMVVGSSPAAAIEILKTHDRNLSARYVPKVLPASQEELNRSSIGWTEVCNDGWKYLRTLCRSELFSIRALDNQSCLREKKVLDMVEHLRAKEGDVVDIGELAFATVFNMLSNVLVSRDLIDLDEERDDGGMKSLVRAIMEVGTAPNISDFYPILCKFDLQGLTKKSIKLGIKVRAVWEPIIEERRQKGVPLSQQDFLDTLLENNFTNVRIHQLLMELFTAGTDTSTSTIEWTMTELVKNPASMKKVREELENEINQDLPKESQVLQLPYLQACIKETLRLHPPAPLLLPHRAPETCQVMNYTIPKNAQILVNVWAIGRDPSIWDEASKFKPERFLSCGLDYKGNDFEFLPFGAGRRICPGLPMAARQVPLVIASLIHCFDWSLPEGKDPQQLDMKESFGFTLQKEQPLLLIPKARK

SEQ ID NO: 54 - protein, 500 aa, Mitragyna speciosa
MELYTLLFCISLLLFIIGPFLHGSSTKKTPPGPKGLPIIGSLLELGSQPHQSLAALAKIHGSIMTLKLGSVTAIIASSPETAKEILQKQEQIFSDRTVPDVVTSQPNPQATLAWVPGDHQWRNKRRICSTQMFTTQRLDLLQHLREKKVEELVLYFKKRSVLGAPVDIGRAAFATTLNLMSNTIFSIDMVDSEFETAQEFKDLVWRIMEDAGKPNLSDYFPVIKWFDLQGVKRHIRPAYRRLHEIFEEVIVERLEDRKLGKRKSRKDDFLDVLLDQCEEEESGFDRETIKPLILDLFIAGSDTSAITTEWAMAELLRKPEAMHKVRTEIIQKIGFERSVKESDVNQLSYLQAVVKETMRLHPAAPLLLPYKANKDTEIFGFTIPKNSQVLVNAWAIGRDPNHWKNSLSFLPERFFGSELDYKGRDFEYIPFGAGRRICPGMPLAVRMVNLMLASIIQAFSWKLPDGITPEKLDMEEQFGVTLKKAVPLCAIPIIEENLGF

SEQ ID NO: 55 - protein, 364 aa, Mitragyna speciosa
MDLARNGDRAGELLQAQAHIWNHIFNFINSMSLKCAVQLGIPDIIEKHGQPMTLAQLCHALSISNTKASFLYRLMRVLIHSGFFIKAKIPGNELEEGYELTSASKLLLKSNPFSVTPFLLAMLAPISTDLWHHFSKWFQSDDETPFHTCHGTSGWEMASQEPWINQSFNEAMASDARLVSSILIEHCGHVFSGLNSLVDVGGGTGTLAKAIADAFPDLKCTVLDLPYVVDGLDGGRKNLAFIGGDIFEAVPPADAVLLKWTLHDWSDEDCVRILEKCKQAIPSKENGGKVIIIDMVINDQQKGADDGEHKSIETQLFFDMLMMVDTKGRERNEKEWAEIFSAAGFKDYKITHALGLRSLIEIYY

SEQ ID NO: 56 - protein, 348 aa, Mitragyna speciosa
MATLENSAELLRAQAHVWSQTFNFKNSASLKCAVQLGIADVIQKHGKPITLSKLAAALPINPSKANYIYRLMRILVNAGFFAQEKEGYSLTSAGRLLLSDEPVNARAFILVVLDPDTIKPWNFLSDWFQNDDPSPFDTAHGKNFWDFTAEEPKFSKLFNEGMVSDSHLITMVLVTECKYVFEGLTSLVDVGGGTGTVARSIAEAFPNLKCTVFDLPHVVANQEGTLNLDFVAGNMLEKVPPANAILLKWILHDWSDEACVKILKNCKKAIPGRDIGGKVIIIDMVMESQLEDDESTEAQICLDMQMLVLYRAKERSEKEWAKLFSDAGFPSYKVFPALGTRAIIEVYP

SEQ ID NO: 57 - protein, 360 aa, Mitragyna speciosa
MDTNDEGSKLLHGQAEIWKHTFRFADSMALKCAAELGIADIIHSHGRPLTLAEIATNITNSSSPHIPYLSRIMRFLVRNKIFTSTDIPSDHGGDSPSTTLYGLTAASRWLLNDNDGLSLAPFLLMENHPWLVSPWHQLSSCVREGGIAFQKAHGKEIWELASENPEFNTIFNDGMGCTGKITMKAILSGFKDAWNTIESLVDVGGGTGQTIAEIVKVYPHIKGINFDLPHVVATAPKYDGVSHVGGDMFDSIPTAQAVLMKWIMHDWGDEDCVKILKICRKAIPEKTGKIFIVDVVLKPDGDGLFDSIGMIFDLLMIAHSSGGKERTEPEWKKLLEKGGFPRYNITEIPACFSIIEAYPV

SEQ ID NO: 58 - protein, 345 aa, Mitragyna speciosa
MEEAKTREEEAQAQVDIWKYIFGFTEMAVVKCAIELGIADVLESREGQAMTLGELSSALGCSPSSLYRIMRFLTNRGIFKQLSGTTYAQTPLSCLLVRNGEKSMAAFVLLESSPVMLAPWHHLRERVSADGPPAFDAAHGQDVWSYAEKNSAHSKLINDAMSCDARFAVSAIIDGCPQVFEGIGSLVDVGGGDGTALRTLLKACPWIRGINFDLPHVVSVTSHCDGVEHVGGDMFDSVPKADAAFIMWVLHDWGDDECISILKNCREAVPQDTGKVIIVEAVTDGGGEDKLKDVGLMLDMVMMAHTTRGKERTSKEWANVLNQAGFSRHTVTRIQAVQSVIEAFP

SEQ ID NO: 59 - protein, 352 aa, Mitragyna speciosa
MGSAEEEASLFAMQLASASVLPMVLKSAIELDLLELIAKAGPGAYVSPSKLAAQLPTHNPQAPVMLDRILRLLATYSVLNCKLRDLPDGGVERLYGLAPVCKFLTKNADGVSMAPLLLMNQDKVLMESWYHLKDAVIDGGIPFNKAYGMTAFEYHGTDPRFNKVFNQGMSNHSTITMKKILEVYKGFEGVKTVVDVGGGTGATLNMIIDKYPTIKGINFELPHVVEDAPFYPGVEHVGGDMFVSVPEGDAIFMKWICHDWSDDHCRKLLKNCYHALPEGGKVILAECILPDAPDTSLATQNVVHIDVIMLAHNPGGKERTEKEFEALAKGAGFKEFRKICSAVNTWIMELCK

SEQ ID NO: 60 - protein, 373 aa, Mitragyna speciosa
MEKEDCLAKTNSNENSEEVVKLGGKVEEEEQLFSYAMQLVTSVSLPRVLLAAFRLRVFEIIAEAGPGAQLSASEIAAQVSGKNKDAAAMLDRMLRLLASHSVLSCGARSQGRVYGLAPVAKYFVQSKADGGGTLGSLLALIQDKVFIDSWYQLEDAVREGGVPFDRVYGTHAFEYPGRDPRFNEVFNKAMLDHTTIAINRILERYKGFENLKTLVDVGGGLGVTLNVITTKYPNLKGINFDLPHVIQRAPGYPGVEHIGGDMFESVPEGEAIFMKWILHDWDDGHCLKLLKNCYKALSDNGKVIVVDALVPVIPDTSPCVKTTCQSDLIMMTQNPGGKERSEPEFLALATAAGFKGIRLECYVCNLWVMEFYK

SEQ ID NO: 61 - protein, 290 aa, Mitragyna speciosa
MEISENAQLKSASPSSIENGQEGEKQDHFSHVMQLVTSASLPMVLYTAVKLNLFEIIAKAGPGAKLSPSEIACRLPTTKNPDAASMLDRMLRLLSSHSLLTYDVVEVAGGAETDIGYERVYGLSPVGEYLIPDEEGNSVAPLVELLLDKVLINTWYELGNAVLEGGIPFNRVHGTHAFDYPSRNPRYNELFNNGMVGPTAITMKELLQQYKGFELLQTLVDVGGGLGITLHKIIAKYPSIRGINFDLPHVIEDAPPYPGMEHIGGDMFESVPGGDAIFMKMILHDWSDDH

SEQ ID NO: 62 - protein, 374 aa, Mitragyna speciosa
MAPTLDTIPTVDVKEMPEEAHPMKGGDDFNSYSQNSCYQRGVIDAAKVVIVEAVNEKLDLKNNANFDPSKPFHIADFGCSTGPNTYFAVQNIVEAVDQKHKSLHEKIQPEFHVFFNDHVNNDFNILFRSLPQDRDYFAAGVPGSFYTRVFPKASVHFAHCSYALHWLSKVPKEIQDKNSPAFNRGRIHYTGTEKHVVKAYFSQFQKDMGSFLKARAQEIVGGGLVVIQIPGLPSGEVLFSRTGAGMLHALLGSSLMELVNLGIISEESVDSFNLPQYHPSIEELEMVIEMNNSFTIEKVGALNHPMKSLPFDVQMTSLQVRAVMEGILSDHFGGKILDQLFEIYTTKLQENYNVFDKEIRRDADLFLVLKRKSN

SEQ ID NO: 63 - protein, 247 aa, Mitragyna speciosa
MAPTVKTPTPIPTPNPNPSLDIKVMPEEAHPMKGGDDLNSYSQNSCYQKGVIDAAKSVIIEAVTEKLDLENNITTFDPAKPFRIADFGCSTGPNTYFAMQNVVEAVELKYKSLKKDQPEFHVFFNDHVNNDFNILFRSLPQNRDYFAAGVPGSFYTRVFPKASLHFAHCSYALHWLSKVPKEIQDKNSPAFNKGGIHYTGTEKHVVKAYFGQFQKDMDSFLKARALEIVGGGLMVIQIPGLPSGEVL

SEQ ID NO: 64 - protein, 389 aa, Mitragyna speciosa
MLQQLPSGFRLQSGAAAEVLAKNRAKMEEGKLVSHTYHMEGGDGPYSYAKNSSYQREAVDSIKEMMNELIAQHLDLGNLYSFRVADFGCSVGPNTFSAVQNIIEAVVNKYKSQGMESQIPEFHVFFNDHAENDFNTLFRNLPTTRGYFPAGVPGSFHRRLLPSSTLYFAHCSTALHWLSKIPKEVMDKNCPAWNKGRIHYAGAAKDVEEAYSTQFGKDLDSFLSARAQELVPGGLLTLVTLGFPDGVQVSDSSMGESFNILGSCFQDMVEEGAIVEELVDSFNLPFYYPSLSELKSLIEVNGLFDIKRLEKLAAPVRREKPDLAVCTLHLRAIIGGLIKEHFGEGIIDNFFERHAKKFVENPIISDERYFKEASFFVFLKRNTTLQCNH

SEQ ID NO: 65 - protein, 375 aa, Mitragyna speciosa
RERERDREEMESVQSNSSSSDQFAMKGGDDDFSYTKNSTHQRDAIQATKFFIQESIAEKLDVNKFCGKAFCVADLGCSVGPNTLIAMQNIVEAVELKFKNRKGFHSPTIPEFQVFFNDHTVNDFNTLFRSLPTGHDKRYYGVGVPGSFYGRLFPCDSIHIMHTSFSTPFLSQVPKEVMDKNSAAWNKGRIHHNYAKADVLKAYEAQHAEDIDCFLTARAKELVHGGLLMDVTSFRPDGVPHTHVLTNIGMEVLGYCLMDLAKKGLIDEENVDSYNVPVYLQSPEELKQAVQRNKYFSIEKMESVPMMIDSDVSAKAQQYSLGMRAVMGDVIREQFGAEIVDKLFDLFKKKLEEHPNFATAVVLDMFVLLKRNAQD